European Patent Application EP 4 230 646 A1, published August 23, 2023. Title: MODIFIED INTERLEUKIN-2 (IL-2) MOLECULE AND USE THEREOF. Applicant: LETO LABORATORIES CO., LTD. The sequence listing filed with the application follows.

SEQUENCE LISTING (26 sequences)

SEQ ID NO: 1 - protein, 24 aa, Homo sapiens
NNYKNPKLTRMLTFKFYMPKKATE

SEQ ID NO: 2 - protein, 20 aa, Homo sapiens
LKHLQCLEEELKPLEEVLNL

SEQ ID NO: 3 - protein, 9 aa, Homo sapiens
AQSKNFHLR

SEQ ID NO: 4 - protein, 16 aa, Homo sapiens
PRDLISNINVIVLELK

SEQ ID NO: 5 - protein, 16 aa, Homo sapiens
GSETTFMCEYADETAT

SEQ ID NO: 6 - protein, 20 aa, Homo sapiens
IVEFLNRWITFCQSIISTLT

SEQ ID NO: 7 - protein, 133 aa, Homo sapiens
APTSSSTKKTQLQLEHLLLDLQMILNGINNYKNPKLTRMLTFKFYMPKKATELKHLQCLEEELKPLEEVLNLAQSKNFHLRPRDLISNINVIVLELKGSETTFMCEYADETATIVEFLNRWITFAQSIISTLT

SEQ ID NO: 8 - protein, 19 aa, Homo sapiens
QSMHIDATLYTESDVHPSC

SEQ ID NO: 9 - protein, 18 aa, Homo sapiens
KVTAMKCFLLELQVISLE

SEQ ID NO: 10 - protein, 5 aa, Homo sapiens
SGDAS

SEQ ID NO: 11 - protein, 16 aa, Homo sapiens
IHDTVENLIILANNSL

SEQ ID NO: 12 - protein, 21 aa, Homo sapiens
SSNGNVTESGCKECEELEEKN

SEQ ID NO: 13 - protein, 114 aa, Homo sapiens
NWVNVISDLKKIEDLIQSMHIDATLYTESDVHPSCKVTAMKCFLLELQVISLESGDASIHDTVENLIILANNSLSSNANVTESGCKECEELEEKNIKEFLQSFVHIVQMFINTS

SEQ ID NO: 14 - protein, 127 aa, Artificial Sequence
  Amino acid sequence of IL-2/IL-15 chimera 1
APTSSSTKKTQLQLEHLLLDLQMILNGIQSMHIDATLYTESDVHPSCKVTAMKCFLLELQVISLESGDASIHDTVENLIILANNSLSSNGNVTESGCKECEELEEKNIVEFLNRFITFAQSIISTLT

SEQ ID NO: 15 - protein, 65 aa, Homo sapiens
ITCPPPMSVEHADIWVKSYSLYSRERYICNSGFKRKAGTSSLTECVLNKATNVAHWTTPSLKCIR

SEQ ID NO: 16 - protein, 175 aa, Homo sapiens
ITCPPPMSVEHADIWVKSYSLYSRERYICNSGFKRKAGTSSLTECVLNKATNVAHWTTPSLKCIRDPALVHQRPAPPSTVTTAGVTPQPESLSPSGKEPAASSPSSNNTAATTAAIVPGSQLMPSKSPSTGTTEISSHESSHGTPSQTTAKNWELTASASHQPPGVYPQGHSDTT

SEQ ID NO: 17 - protein, 219 aa, Homo sapiens
ELCDDDPPEIPHATFKAMAYKEGTMLNCECKRGFRRIKSGSLYMLCTGNSSHSSWDNQCQCTSSATRNTTKQVTPQPEEQKERKTTEMQSPMQPVDQASLPGHCREPPPWENEATERIYHFVVGQMVYYQCVQGYRALHRGPAESVCKMTHGKTRWTQPQLICTGEMETSQFPGEEKPQASPEGRPESETSCLVTTTDFQIQTEMAATMETSIFTTEYQ

SEQ ID NO: 18 - protein, 232 aa, Homo sapiens
EPKSCDKTHTCPPCPAPELLGGPSVFLFPPKPKDTLMISRTPEVTCVVVDVSHEDPEVKFNWYVDGVEVHNAKTKPREEQYNSTYRVVSVLTVLHQDWLNGKEYKCKVSNKALPAPIEKTISKAKGQPREPQVYTLPPSRDELTKNQVSLTCLVKGFYPSDIAVEWESNGQPENNYKTTPPVLDSDGSFFLYSKLTVDKSRWQQGNVFSCSVMHEALHNHYTQKSLSLSPGK

SEQ ID NO: 19 - protein, 297 aa, Artificial Sequence
  Amino acid sequence of Sushi-hlgG1Fc
ITCPPPMSVEHADIWVKSYSLYSRERYICNSGFKRKAGTSSLTECVLNKATNVAHWTTPSLKCIREPKSCDKTHTCPPCPAPELLGGPSVFLFPPKPKDTLMISRTPEVTCVVVDVSHEDPEVKFNWYVDGVEVHNAKTKPREEQYNSTYRVVSVLTVLHQDWLNGKEYKCKVSNKALPAPIEKTISKAKGQPREPQVYTLPPSRDELTKNQVSLTCLVKGFYPSDIAVEWESNGQPENNYKTTPPVLDSDGSFFLYSKLTVDKSRWQQGNVFSCSVMHEALHNHYTQKSLSLSPGK

SEQ ID NO: 20 - protein, 78 aa, Homo sapiens
ITCPPPMSVEHADIWVKSYSLYSRERYICNSGFKRKAGTSSLTECVLNKATNVAHWTTPSLKCIRDPALVHQRPAPPS

SEQ ID NO: 21 - protein, 293 aa, Artificial Sequence
  Amino acid sequence of Sushi-hIgG4Fc
ITCPPPMSVEHADIWVKSYSLYSRERYICNSGFKRKAGTSSLTECVLNKATNVAHWTTPSLKCIRESKYGPPCPPCPAPEFLGGPSVFLFPPKPKDTLMISRTPEVTCVVVDVSQEDPEVQFNWYVDGVEVHNAKTKPREEQFNSTYRVVSVLTVLHQDWLNGKEYKCKVSNKGLPSSIEKTISKAKGQPREPQVYTLPPSQEEMTKNQVSLTCLVKGFYPSDIAVEWESNGQPENNYKTTPPVLDSDGSFFLYSRLTVDKSRWQEGNVFSCSVMHEALHNHYTQKSLSLSLG

SEQ ID NO: 22 - protein, 298 aa, Artificial Sequence
  Amino acid sequence of Sushi-mlgG2aa.1Fc
ITCPPPMSVEHADIWVKSYSLYSRERYICNSGFKRKAGTSSLTECVLNKATNVAHWTTPSLKCIREPRGPTIKPCPPCKCPAPNAEGAPSVFIFPPKIKDVLMISLSPIVTCVVVDVSEDDPDVQISWFVNNVEVHTAQTQTHREDYNSTLRVVSALPIQHQDWMSGKEFKCKVNNKQLPSSIERTISKPKGSVRAPQVYVLPPPEEEMTKKQVTLTCMVTDFMPEDIYVEWTNNGKTELNYKNTEPVLDSDGSYFMYSKLRVEKKNWVERNSYSCSVVHEGLHNHHTTKSFSRTPGK

SEQ ID NO: 23 - protein, 127 aa, Artificial Sequence
  Amino acid sequence of IL-2/15 chimera 2
APTSSSTKKTQLQLEHLLLDLQMILNGIQSMHIDATLYTESDVHPSCKVTAMKCFLLELQVISLESGDASIHDTVENLIILANNSLSSNGNVTESGCKECEELEEKNIVEFLNRWITFAQSIISTLT

SEQ ID NO: 24 - protein, 228 aa, Homo sapiens
ESKYGPPCPPCPAPEFLGGPSVFLFPPKPKDTLMISRTPEVTCVVVDVSQEDPEVQFNWYVDGVEVHNAKTKPREEQFNSTYRVVSVLTVLHQDWLNGKEYKCKVSNKGLPSSIEKTISKAKGQPREPQVYTLPPSQEEMTKNQVSLTCLVKGFYPSDIAVEWESNGQPENNYKTTPPVLDSDGSFFLYSRLTVDKSRWQEGNVFSCSVMHEALHNHYTQKSLSLSLG

SEQ ID NO: 25 - protein, 233 aa, Homo sapiens
EPRGPTIKPCPPCKCPAPNAEGAPSVFIFPPKIKDVLMISLSPIVTCVVVDVSEDDPDVQISWFVNNVEVHTAQTQTHREDYNSTLRVVSALPIQHQDWMSGKEFKCKVNNKQLPSSIERTISKPKGSVRAPQVYVLPPPEEEMTKKQVTLTCMVTDFMPEDIYVEWTNNGKTELNYKNTEPVLDSDGSYFMYSKLRVEKKNWVERNSYSCSVVHEGLHNHHTTKSFSRTPGK

SEQ ID NO: 26 - DNA, 381 bp, Artificial Sequence
  Amino acid sequence of synthesized IL-2/15 chimera 1
gcgccgacgagcagtagcaccaaaaaaacgcagctgcagctggaacatctgttactggatctgcagatgattctgaacggcattcagagcatgcatattgatgcgaccctgtataccgaaagcgatgtgcatccgagctgcaaagtgaccgcgatgaaatgctttctgctggaactgcaagtgattagcctggaaagcggcgatgcgagcattcatgataccgtggaaaacctgattattctggcgaacaacagcctgagcagcaacggcaacgtgaccgaaagcggctgcaaagaatgcgaagaactggaagaaaaaaacattgtggaatttctgaaccgctttattacctttgcgcagagcattattagcaccctgacc